European Patent Specification EP 3 999 651 B1, published March 18, 2026. Title: METHODS OF PERFORMING GUIDE-SEQ ON PRIMARY HUMAN T CELLS. Applicant: PACT PHARMA, INC. The sequence listing filed with the application follows.

SEQUENCE LISTING (11 sequences)

SEQ ID NO: 1 - DNA, 34 bp, Artificial Sequence
  Synthetic polynucleotide
  modified_base (1)..(1): 5Phos-g
  misc_feature (1)..(3): Phosphorothioate linkage
  misc_feature (32)..(34): Phosphorothioate linkage
gtttaattgagttgtcatatgttaataacggtat

SEQ ID NO: 2 - DNA, 34 bp, Artificial Sequence
  Synthetic polynucleotide
  modified_base (1)..(1): 5Phos-a
  misc_feature (1)..(3): Phosphorothioate linkage
  misc_feature (32)..(34): Phosphorothioate linkage
ataccgttattaacatatgacaactcaattaaac

SEQ ID NO: 3 - DNA, 20 bp, Artificial Sequence
  Synthetic polynucleotide
tcacgagcagctggtttcta

SEQ ID NO: 4 - DNA, 20 bp, Artificial Sequence
  Synthetic polynucleotide
gggttttggtggcaatggat

SEQ ID NO: 5 - DNA, 20 bp, Artificial Sequence
  Synthetic polynucleotide
caacagacactgggatggtg

SEQ ID NO: 6 - DNA, 20 bp, Artificial Sequence
  Synthetic polynucleotide
gctctgttgggctgagaatc

SEQ ID NO: 7 - DNA, 20 bp, Artificial Sequence
  Synthetic polynucleotide
ctaactgggggatggacaga

SEQ ID NO: 8 - DNA, 20 bp, Artificial Sequence
  Synthetic polynucleotide
gagcttgaggtgctccattc

SEQ ID NO: 9 - DNA, 23 bp, Artificial Sequence
  Synthetic polynucleotide
  misc_feature (21)..(21): n is a, c, g, or t
gagaatcaaaatcggtgaatngg

SEQ ID NO: 10 - DNA, 23 bp, Artificial Sequence
  Synthetic polynucleotide
gagaatcaaaatcggtgaatagg

SEQ ID NO: 11 - DNA, 23 bp, Artificial Sequence
  Synthetic polynucleotide
gagaatcaaaatcggtgaatagg